European Patent Application EP 4 516 800 A2, published March 5, 2025. Title: ANTI-VEGF PROTEIN COMPOSITIONS AND METHODS FOR PRODUCING THE SAME. Applicant: REGENERON PHARMACEUTICALS, INC. Application EP Divisional of European patent application no. 20764873.4, filed August 18, 2020. The sequence listing filed with the application follows.

SEQUENCE LISTING (103 sequences)

SEQ ID NO: 1 - protein, 339 aa, synthetic construct
  REGION 1..339: note = source = /note="Description of Artificial Sequence: Synthetic polypeptide"
MRKRCYSTSAAVLAAVTLFVLSVDRGVIADSFSANQEIRYSEVTPYHVTSVWTKGVTPPANFTQGEDVFHAPYVANQGWYDITKTFNGKDDLLCGAATAGNMLHWWFDQNKDQIKRYLEEHPEKQKINFNGEQMFDVKEAIDTKNHQLDSKLFEYFKEKAFPYLSTKHLGVFPDHVIDMFINGYRLSLTNHGPTPVKEGSKDPRGGIFDAVFTRGDQSKLLTSRHDFKEKNLKEISDLIKKELTEGKALGLSHTYANVRINHVINLWGADFDSNGNLKAIYVTDSDSNASIGMKKYFVGVNSAGKVAISAKEIKEDNIGAQVLGLFTLSTGQDSWNQTN

SEQ ID NO: 2 - protein, 339 aa, synthetic construct
  REGION 1..339: note = source = /note="Description of Artificial Sequence: Synthetic polypeptide"
MRKRCYSTSAAVLAAVTLFVLSVDRGVIADSFSANQEIRYSEVTPYHVTSVWTKGVTPPANFTQGEDVFHAPYVANQGWYDITKTFDGKDDLLCGAATAGNMLHWWFDQNKDQIKRYLEEHPEKQKINFNGEQMFDVKEAIDTKNHQLDSKLFEYFKEKAFPYLSTKHLGVFPDHVIDMFINGYRLSLTNHGPTPVKEGSKDPRGGIFDAVFTRGDQSKLLTSRHDFKEKNLKEISDLIKKELTEGKALGLSHTYANVRINHVINLWGADFDSNGNLKAIYVTDSDSNASIGMKKYFVGVNSAGKVAISAKEIKEDNIGAQVLGLFTLSTGQDSWNQTN

SEQ ID NO: 3 - protein, 339 aa, synthetic construct
  REGION 1..339: note = source = /note="Description of Artificial Sequence: Synthetic polypeptide"
MRKRCYSTSAAVLAAVTLFVLSVDRGVIADSFSANQEIRYSEVTPYHVTSVWTKGVTPPANFTQGEDVFHAPYVANQGWYDITKTFNGKDDLLCGAATAGNMLHWWFDQNKDQIKRYLEEHPEKQKINFRGEQMFDVKEAIDTKNHQLDSKLFEYFKEKAFPYLSTKHLGVFPDHVIDMFINGYRLSLTNHGPTPVKEGSKDPRGGIFDAVFTRGDQSKLLTSRHDFKEKNLKEISDLIKKELTEGKALGLSHTYANVRINHVINLWGADFDSNGNLKAIYVTDSDSNASIGMKKYFVGVNSAGKVAISAKEIKEDNIGAQVLGLFTLSTGQDSWNQTN

SEQ ID NO: 4 - protein, 339 aa, synthetic construct
  REGION 1..339: note = source = /note="Description of Artificial Sequence: Synthetic polypeptide"
MRKRCYSTSAAVLAAVTLFVLSVDRGVIADSFSANQEIRYSEVTPYHVTSVWTKGVTPPANFTQGEDVFHAPYVANQGWYDITKTFNGKDDLLCGAATAGNMLHWWFDQNKDQIKRYLEEHPEKQKINFNGEQMFDVKEAIDTKNHQLDSKLFEYFKEKAFPYLSTKHLGVFPDHVIDMFILGYRLSLTNHGPTPVKEGSKDPRGGIFDAVFTRGDQSKLLTSRHDFKEKNLKEISDLIKKELTEGKALGLSHTYANVRINHVINLWGADFDSNGNLKAIYVTDSDSNASIGMKKYFVGVNSAGKVAISAKEIKEDNIGAQVLGLFTLSTGQDSWNQTN

SEQ ID NO: 5 - protein, 339 aa, synthetic construct
  REGION 1..339: note = source = /note="Description of Artificial Sequence: Synthetic polypeptide"
MRKRCYSTSAAVLAAVTLFVLSVDRGVIADSFSANQEIRYSEVTPYHVTSVWTKGVTPPANFTQGEDVFHAPYVANQGWYDITKTFNGKDDLLCGAATAGNMLHWWFDQNKDQIKRYLEEHPEKQKINFNGEQMFDVKEAIDTKNHQLDSKLFEYFKEKAFPYLSTKHLGVFPDHVIDMFINGYRLSLTNHGPTPVKEGSKDPRGGIFDAVFTRGDQSKLLTSRHDFKEKNLKEISDLIKKELTEGKALGLSHTYANVRINHVINLWGADFDSDGNLKAIYVTDSDSNASIGMKKYFVGVNSAGKVAISAKEIKEDNIGAQVLGLFTLSTGQDSWNQTN

SEQ ID NO: 6 - protein, 339 aa, synthetic construct
  REGION 1..339: note = source = /note="Description of Artificial Sequence: Synthetic polypeptide"
MRKRCYSTSAAVLAAVTLFVLSVDRGVIADSFSANQEIRYSEVTPYHVTSVWTKGVTPPANFTQGEDVFHAPYVANQGWYDITKTFDGKDDLLCGAATAGNMLHWWFDQNKDQIKRYLEEHPEKQKINFRGEQMFDVKEAIDTKNHQLDSKLFEYFKEKAFPYLSTKHLGVFPDHVIDMFINGYRLSLTNHGPTPVKEGSKDPRGGIFDAVFTRGDQSKLLTSRHDFKEKNLKEISDLIKKELTEGKALGLSHTYANVRINHVINLWGADFDSNGNLKAIYVTDSDSNASIGMKKYFVGVNSAGKVAISAKEIKEDNIGAQVLGLFTLSTGQDSWNQTN

SEQ ID NO: 7 - protein, 339 aa, synthetic construct
  REGION 1..339: note = source = /note="Description of Artificial Sequence: Synthetic polypeptide"
MRKRCYSTSAAVLAAVTLFVLSVDRGVIADSFSANQEIRYSEVTPYHVTSVWTKGVTPPANFTQGEDVFHAPYVANQGWYDITKTFDGKDDLLCGAATAGNMLHWWFDQNKDQIKRYLEEHPEKQKINFNGEQMFDVKEAIDTKNHQLDSKLFEYFKEKAFPYLSTKHLGVFPDHVIDMFILGYRLSLTNHGPTPVKEGSKDPRGGIFDAVFTRGDQSKLLTSRHDFKEKNLKEISDLIKKELTEGKALGLSHTYANVRINHVINLWGADFDSNGNLKAIYVTDSDSNASIGMKKYFVGVNSAGKVAISAKEIKEDNIGAQVLGLFTLSTGQDSWNQTN

SEQ ID NO: 8 - protein, 339 aa, synthetic construct
  REGION 1..339: note = source = /note="Description of Artificial Sequence: Synthetic polypeptide"
MRKRCYSTSAAVLAAVTLFVLSVDRGVIADSFSANQEIRYSEVTPYHVTSVWTKGVTPPANFTQGEDVFHAPYVANQGWYDITKTFDGKDDLLCGAATAGNMLHWWFDQNKDQIKRYLEEHPEKQKINFNGEQMFDVKEAIDTKNHQLDSKLFEYFKEKAFPYLSTKHLGVFPDHVIDMFINGYRLSLTNHGPTPVKEGSKDPRGGIFDAVFTRGDQSKLLTSRHDFKEKNLKEISDLIKKELTEGKALGLSHTYANVRINHVINLWGADFDSDGNLKAIYVTDSDSNASIGMKKYFVGVNSAGKVAISAKEIKEDNIGAQVLGLFTLSTGQDSWNQTN

SEQ ID NO: 9 - protein, 339 aa, synthetic construct
  REGION 1..339: note = source = /note="Description of Artificial Sequence: Synthetic polypeptide"
MRKRCYSTSAAVLAAVTLFVLSVDRGVIADSFSANQEIRYSEVTPYHVTSVWTKGVTPPANFTQGEDVFHAPYVANQGWYDITKTFNGKDDLLCGAATAGNMLHWWFDQNKDQIKRYLEEHPEKQKINFRGEQMFDVKEAIDTKNHQLDSKLFEYFKEKAFPYLSTKHLGVFPDHVIDMFILGYRLSLTNHGPTPVKEGSKDPRGGIFDAVFTRGDQSKLLTSRHDFKEKNLKEISDLIKKELTEGKALGLSHTYANVRINHVINLWGADFDSNGNLKAIYVTDSDSNASIGMKKYFVGVNSAGKVAISAKEIKEDNIGAQVLGLFTLSTGQDSWNQTN

SEQ ID NO: 10 - protein, 339 aa, synthetic construct
  REGION 1..339: note = source = /note="Description of Artificial Sequence: Synthetic polypeptide"
MRKRCYSTSAAVLAAVTLFVLSVDRGVIADSFSANQEIRYSEVTPYHVTSVWTKGVTPPANFTQGEDVFHAPYVANQGWYDITKTFNGKDDLLCGAATAGNMLHWWFDQNKDQIKRYLEEHPEKQKINFRGEQMFDVKEAIDTKNHQLDSKLFEYFKEKAFPYLSTKHLGVFPDHVIDMFINGYRLSLTNHGPTPVKEGSKDPRGGIFDAVFTRGDQSKLLTSRHDFKEKNLKEISDLIKKELTEGKALGLSHTYANVRINHVINLWGADFDSDGNLKAIYVTDSDSNASIGMKKYFVGVNSAGKVAISAKEIKEDNIGAQVLGLFTLSTGQDSWNQTN

SEQ ID NO: 11 - protein, 339 aa, synthetic construct
  REGION 1..339: note = source = /note="Description of Artificial Sequence: Synthetic polypeptide"
MRKRCYSTSAAVLAAVTLFVLSVDRGVIADSFSANQEIRYSEVTPYHVTSVWTKGVTPPANFTQGEDVFHAPYVANQGWYDITKTFNGKDDLLCGAATAGNMLHWWFDQNKDQIKRYLEEHPEKQKINFNGEQMFDVKEAIDTKNHQLDSKLFEYFKEKAFPYLSTKHLGVFPDHVIDMFILGYRLSLTNHGPTPVKEGSKDPRGGIFDAVFTRGDQSKLLTSRHDFKEKNLKEISDLIKKELTEGKALGLSHTYANVRINHVINLWGADFDSDGNLKAIYVTDSDSNASIGMKKYFVGVNSAGKVAISAKEIKEDNIGAQVLGLFTLSTGQDSWNQTN

SEQ ID NO: 12 - protein, 339 aa, synthetic construct
  REGION 1..339: note = source = /note="Description of Artificial Sequence: Synthetic polypeptide"
MRKRCYSTSAAVLAAVTLFVLSVDRGVIADSFSANQEIRYSEVTPYHVTSVWTKGVTPPANFTQGEDVFHAPYVANQGWYDITKTFDGKDDLLCGAATAGNMLHWWFDQNKDQIKRYLEEHPEKQKINFRGEQMFDVKEAIDTKNHQLDSKLFEYFKEKAFPYLSTKHLGVFPDHVIDMFILGYRLSLTNHGPTPVKEGSKDPRGGIFDAVFTRGDQSKLLTSRHDFKEKNLKEISDLIKKELTEGKALGLSHTYANVRINHVINLWGADFDSNGNLKAIYVTDSDSNASIGMKKYFVGVNSAGKVAISAKEIKEDNIGAQVLGLFTLSTGQDSWNQTN

SEQ ID NO: 13 - protein, 339 aa, synthetic construct
  REGION 1..339: note = source = /note="Description of Artificial Sequence: Synthetic polypeptide"
MRKRCYSTSAAVLAAVTLFVLSVDRGVIADSFSANQEIRYSEVTPYHVTSVWTKGVTPPANFTQGEDVFHAPYVANQGWYDITKTFDGKDDLLCGAATAGNMLHWWFDQNKDQIKRYLEEHPEKQKINFRGEQMFDVKEAIDTKNHQLDSKLFEYFKEKAFPYLSTKHLGVFPDHVIDMFINGYRLSLTNHGPTPVKEGSKDPRGGIFDAVFTRGDQSKLLTSRHDFKEKNLKEISDLIKKELTEGKALGLSHTYANVRINHVINLWGADFDSDGNLKAIYVTDSDSNASIGMKKYFVGVNSAGKVAISAKEIKEDNIGAQVLGLFTLSTGQDSWNQTN

SEQ ID NO: 14 - protein, 339 aa, synthetic construct
  REGION 1..339: note = source = /note="Description of Artificial Sequence: Synthetic polypeptide"
MRKRCYSTSAAVLAAVTLFVLSVDRGVIADSFSANQEIRYSEVTPYHVTSVWTKGVTPPANFTQGEDVFHAPYVANQGWYDITKTFDGKDDLLCGAATAGNMLHWWFDQNKDQIKRYLEEHPEKQKINFNGEQMFDVKEAIDTKNHQLDSKLFEYFKEKAFPYLSTKHLGVFPDHVIDMFILGYRLSLTNHGPTPVKEGSKDPRGGIFDAVFTRGDQSKLLTSRHDFKEKNLKEISDLIKKELTEGKALGLSHTYANVRINHVINLWGADFDSDGNLKAIYVTDSDSNASIGMKKYFVGVNSAGKVAISAKEIKEDNIGAQVLGLFTLSTGQDSWNQTN

SEQ ID NO: 15 - protein, 339 aa, synthetic construct
  REGION 1..339: note = source = /note="Description of Artificial Sequence: Synthetic polypeptide"
MRKRCYSTSAAVLAAVTLFVLSVDRGVIADSFSANQEIRYSEVTPYHVTSVWTKGVTPPANFTQGEDVFHAPYVANQGWYDITKTFNGKDDLLCGAATAGNMLHWWFDQNKDQIKRYLEEHPEKQKINFRGEQMFDVKEAIDTKNHQLDSKLFEYFKEKAFPYLSTKHLGVFPDHVIDMFILGYRLSLTNHGPTPVKEGSKDPRGGIFDAVFTRGDQSKLLTSRHDFKEKNLKEISDLIKKELTEGKALGLSHTYANVRINHVINLWGADFDSDGNLKAIYVTDSDSNASIGMKKYFVGVNSAGKVAISAKEIKEDNIGAQVLGLFTLSTGQDSWNQTN

SEQ ID NO: 16 - protein, 339 aa, synthetic construct
  REGION 1..339: note = source = /note="Description of Artificial Sequence: Synthetic polypeptide"
MRKRCYSTSAAVLAAVTLFVLSVDRGVIADSFSANQEIRYSEVTPYHVTSVWTKGVTPPANFTQGEDVFHAPYVANQGWYDITKTFDGKDDLLCGAATAGNMLHWWFDQNKDQIKRYLEEHPEKQKINFRGEQMFDVKEAIDTKNHQLDSKLFEYFKEKAFPYLSTKHLGVFPDHVIDMFILGYRLSLTNHGPTPVKEGSKDPRGGIFDAVFTRGDQSKLLTSRHDFKEKNLKEISDLIKKELTEGKALGLSHTYANVRINHVINLWGADFDSDGNLKAIYVTDSDSNASIGMKKYFVGVNSAGKVAISAKEIKEDNIGAQVLGLFTLSTGQDSWNQTN

SEQ ID NO: 17 - protein, 16 aa, synthetic construct
  REGION 1..16: note = source = /note="Description of Artificial Sequence: Synthetic peptide"
DKTHTCPPCPAPELLG

SEQ ID NO: 18 - protein, 17 aa, synthetic construct
  REGION 1..17: note = source = /note="Description of Artificial Sequence: Synthetic peptide"
EIGLLTCEATVNGHLYK

SEQ ID NO: 19 - protein, 23 aa, synthetic construct
  REGION 1..23: note = source = /note="Description of Artificial Sequence: Synthetic peptide"
QTNTIIDVVLSPSHGIELSVGEK

SEQ ID NO: 20 - protein, 21 aa, synthetic construct
  REGION 1..21: note = source = /note="Description of Artificial Sequence: Synthetic peptide"
TELNVGIDFNWEYPSSKHQHK

SEQ ID NO: 21 - protein, 7 aa, synthetic construct
  REGION 1..7: note = source = /note="Description of Artificial Sequence: Synthetic peptide"
TNYLTHR

SEQ ID NO: 22 - protein, 24 aa, synthetic construct
  REGION 1..24: note = source = /note="Description of Artificial Sequence: Synthetic peptide"
SDTGRPFVEMYSEIPEIIHMTEGR

SEQ ID NO: 23 - protein, 6 aa, synthetic construct
  REGION 1..6: note = source = /note="Description of Artificial Sequence: Synthetic peptide"
VHEKDK

SEQ ID NO: 24 - protein, 24 aa, synthetic construct
  REGION 1..24: note = source = /note="Description of Artificial Sequence: Synthetic peptide"
SDTGRPFVEMYSEIPEIIHMTEGR

SEQ ID NO: 25 - protein, 24 aa, synthetic construct
  REGION 1..24: note = source = /note="Description of Artificial Sequence: Synthetic peptide"
SDTGRPFVEMYSEIPEIIHMTEGR

SEQ ID NO: 26 - protein, 8 aa, synthetic construct
  REGION 1..8: note = source = /note="Description of Artificial Sequence: Synthetic peptide"
TQSGSEMK

SEQ ID NO: 27 - protein, 17 aa, synthetic construct
  REGION 1..17: note = source = /note="Description of Artificial Sequence: Synthetic peptide"
SDQGLYTCAASSGLMTK

SEQ ID NO: 28 - protein, 6 aa, synthetic construct
  REGION 1..6: note = source = /note="Description of Artificial Sequence: Synthetic peptide"
IIWDSR

SEQ ID NO: 29 - protein, 17 aa, synthetic construct
  REGION 1..17: note = source = /note="Description of Artificial Sequence: Synthetic peptide"
TELNVGIDFNWEYPSSK

SEQ ID NO: 30 - protein, 10 aa, synthetic construct
  REGION 1..10: note = source = /note="Description of Artificial Sequence: Synthetic peptide"
GFIISNATYK

SEQ ID NO: 31 - protein, 12 aa, synthetic construct
  REGION 1..12: note = source = /note="Description of Artificial Sequence: Synthetic peptide"
KFPLDTLIPDGK

SEQ ID NO: 32 - protein, 12 aa, synthetic construct
  REGION 1..12: note = source = /note="Description of Artificial Sequence: Synthetic peptide"
FLSTLTIDGVTR

SEQ ID NO: 33 - protein, 227 aa, synthetic construct
  VARIANT 8: note = /replace="Pro"
  VARIANT 173: note = /replace="Thr"
  SITE 1..227: note = /note="Variant residues given in the sequence have no preference with respect to those in the annotations for variant positions"
  REGION 1..227: note = source = /note="Description of Artificial Sequence: Synthetic polypeptide"
DKTHTCPLCPAPELLGGPSVFLFPPKPKDTLMISRTPEVTCVVVDVSHEDPEVKFNWYVDGVEVHNAKTKPREEQYNSTYRVVSVLTVLHQDWLNGKEYKCKVSNKALPAPIEKTISKAKGQPREPQVYTLPPSRDELTKNQVSLTCLVKGFYPSDIAVEWESNGQPENNYKATPPVLDSDGSFFLYSKLTVDKSRWQQGNVFSCSVMHEALHNHYTQKSLSLSPGK

SEQ ID NO: 34 - protein, 103 aa, synthetic construct
  REGION 1..103: note = source = /note="Description of Artificial Sequence: Synthetic polypeptide"
SDTGRPFVEMYSEIPEIIHMTEGRELVIPCRVTSPNITVTLKKFPLDTLIPDGKRIIWDSRKGFIISNATYKEIGLLTCEATVNGHLYKTNYLTHRQTNTIID

SEQ ID NO: 35 - protein, 93 aa, synthetic construct
  REGION 1..93: note = source = /note="Description of Artificial Sequence: Synthetic polypeptide"
PFVEMYSEIPEIIHMTEGRELVIPCRVTSPNITVTLKKFPLDTLIPDGKRIIWDSRKGFIISNATYKEIGLLTCEATVNGHLYKTNYLTHRQT

SEQ ID NO: 36 - protein, 102 aa, synthetic construct
  REGION 1..102: note = source = /note="Description of Artificial Sequence: Synthetic polypeptide"
VVLSPSHGIELSVGEKLVLNCTARTELNVGIDFNWEYPSSKHQHKKLVNRDLKTQSGSEMKKFLSTLTIDGVTRSDQGLYTCAASSGLMTKKNSTFVRVHEK

SEQ ID NO: 37 - protein, 97 aa, synthetic construct
  REGION 1..97: note = source = /note="Description of Artificial Sequence: Synthetic polypeptide"
PFVAFGSGMESLVEATVGERVRIPAKYLGYPPPEIKWYKNGIPLESNHTIKAGHVLTIMEVSERDTGNYTVILTNPISKEKQSHVVSLVVYVPPGPG

SEQ ID NO: 38 - protein, 92 aa, synthetic construct
  REGION 1..92: note = source = /note="Description of Artificial Sequence: Synthetic polypeptide"
FVAFGSGMESLVEATVGERVRIPAKYLGYPPPEIKWYKNGIPLESNHTIKAGHVLTIMEVSERDTGNYTVILTNPIKSEKQSHVVSLVVYVP

SEQ ID NO: 39 - protein, 9 aa, synthetic construct
  REGION 1..9: note = source = /note="Description of Artificial Sequence: Synthetic peptide"
DKTHTCPPC

SEQ ID NO: 40 - protein, 12 aa, synthetic construct
  REGION 1..12: note = source = /note="Description of Artificial Sequence: Synthetic peptide"
DKTHTCPPCPPC

SEQ ID NO: 41 - protein, 15 aa, synthetic construct
  REGION 1..15: note = source = /note="Description of Artificial Sequence: Synthetic peptide"
DKTHTCPPCPPCPPC

SEQ ID NO: 42 - protein, 16 aa, synthetic construct
  REGION 1..16: note = source = /note="Description of Artificial Sequence: Synthetic peptide"
DKTHTCPPCPAPELLG

SEQ ID NO: 43 - protein, 16 aa, synthetic construct
  REGION 1..16: note = source = /note="Description of Artificial Sequence: Synthetic peptide"
DKTHTCPLCPAPELLG

SEQ ID NO: 44 - protein, 6 aa, synthetic construct
  REGION 1..6: note = source = /note="Description of Artificial Sequence: Synthetic peptide"
DKTHTC

SEQ ID NO: 45 - protein, 12 aa, synthetic construct
  REGION 1..12: note = source = /note="Description of Artificial Sequence: Synthetic peptide"
DKTHTCPLCPAP

SEQ ID NO: 46 - protein, 221 aa, synthetic construct
  REGION 1..221: note = source = /note="Description of Artificial Sequence: Synthetic polypeptide"
SDTGRPFVEMYSEIPEIIHMTEGRELVIPCRVTSPNITVTLKKFPLDTLIPDGKRIIWDSRKGFIISNATYKEIGLLTCEATVNGHLYKTNYLTHRQTNTIIDVVLSPSHGIELSVGEKLVLNCTARTELNVGIDFNWEYPSSKHQHKKLVNRDLKTQSGSEMKKFLSTLTIDGVTRSDQGLYTCAASSGLMTKKNSTFVRVHEKDKTHTCPPCPAPELLG

SEQ ID NO: 47 - protein, 315 aa, synthetic construct
  REGION 1..315: note = source = /note="Description of Artificial Sequence: Synthetic polypeptide"
GRPFVEMYSEIPEIIHMTEGRELVIPCRVTSPNITVTLKKFPLDTLIPDGKRIIWDSRKGFIISNATYKEIGLLTCEATVNGHLYKTNYLTHRQTNTIIDVVLSPSHGIELSVGEKLVLNCTARTELNVGIDFNWEYPSSKHQHKKLVNRDLKTQSGSEMKKFLSTLTIDGVTRSDQGLYTCAASSGLMTKKNSTFVRVHENLSVAFGSGMESLVEATVGERVRIPAKYLGYPPPEIKWYKNGIPLESNHTIKAGHVLTIMEVSERDTGNYTVILTNPISKEKQSHVVSLVVYVPPGPGDKTHTCPLCPAPELLG

SEQ ID NO: 48 - protein, 214 aa, synthetic construct
  REGION 1..214: note = source = /note="Description of Artificial Sequence: Synthetic polypeptide"
SDTGRPFVEMYSEIPEIIHMTEGRELVIPCRVTSPNITVTLKKFPLDTLIPDGKRIIWDSRKGFIISNATYKEIGLLTCEATVNGHLYKTNYLTHRQTNTIIDVVLSPSHGIELSVGEKLVLNCTARTELNVGIDFNWEYPSSKHQHKKLVNRDLKTQSGSEMKKFLSTLTIDGVTRSDQGLYTCAASSGLMTKKNSTFVRVHEKDKTHTCPPC

SEQ ID NO: 49 - protein, 217 aa, synthetic construct
  REGION 1..217: note = source = /note="Description of Artificial Sequence: Synthetic polypeptide"
SDTGRPFVEMYSEIPEIIHMTEGRELVIPCRVTSPNITVTLKKFPLDTLIPDGKRIIWDSRKGFIISNATYKEIGLLTCEATVNGHLYKTNYLTHRQTNTIIDVVLSPSHGIELSVGEKLVLNCTARTELNVGIDFNWEYPSSKHQHKKLVNRDLKTQSGSEMKKFLSTLTIDGVTRSDQGLYTCAASSGLMTKKNSTFVRVHEKDKTHTCPPCPPC

SEQ ID NO: 50 - protein, 220 aa, synthetic construct
  REGION 1..220: note = source = /note="Description of Artificial Sequence: Synthetic polypeptide"
SDTGRPFVEMYSEIPEIIHMTEGRELVIPCRVTSPNITVTLKKFPLDTLIPDGKRIIWDSRKGFIISNATYKEIGLLTCEATVNGHLYKTNYLTHRQTNTIIDVVLSPSHGIELSVGEKLVLNCTARTELNVGIDFNWEYPSSKHQHKKLVNRDLKTQSGSEMKKFLSTLTIDGVTRSDQGLYTCAASSGLMTKKNSTFVRVHEKDKTHTCPPCPPCPPC

SEQ ID NO: 51 - protein, 440 aa, synthetic construct
  REGION 1..440: note = source = /note="Description of Artificial Sequence: Synthetic polypeptide"
SDTGRPFVEMYSEIPEIIHMTEGRELVIPCRVTSPNITVTLKKFPLDTLIPDGKRIIWDSRKGFIISNATYKEIGLLTCEATVNGHLYKTNYLTHRQTNTIIDVVLSPSHGIELSVGEKLVLNCTARTELNVGIDFNWEYPSSKHQHKKLVNRDLKTQSGSEMKKFLSTLTIDGVTRSDQGLYTCAASSGLMTKKNSTFVRVHEKGGGGSGGGGSGGGGSGGGGSGGGGSGGGGSSDTGRPFVEMYSEIPEIIHMTEGRELVIPCRVTSPNITVTLKKFPLDTLIPDGKRIIWDSRKGFIISNATYKEIGLLTCEATVNGHLYKTNYLTHRQTNTIIDVVLSPSHGIELSVGEKLVLNCTARTELNVGIDFNWEYPSSKHQHKKLVNRDLKTQSGSEMKKFLSTLTIDGVTRSDQGLYTCAASSGLMTKKNSTFVRVHEK

SEQ ID NO: 52 - protein, 425 aa, synthetic construct
  REGION 1..425: note = source = /note="Description of Artificial Sequence: Synthetic polypeptide"
SDTGRPFVEMYSEIPEIIHMTEGRELVIPCRVTSPNITVTLKKFPLDTLIPDGKRIIWDSRKGFIISNATYKEIGLLTCEATVNGHLYKTNYLTHRQTNTIIDVVLSPSHGIELSVGEKLVLNCTARTELNVGIDFNWEYPSSKHQHKKLVNRDLKTQSGSEMKKFLSTLTIDGVTRSDQGLYTCAASSGLMTKKNSTFVRVHEKGGGGSGGGGSGGGGSSDTGRPFVEMYSEIPEIIHMTEGRELVIPCRVTSPNITVTLKKFPLDTLIPDGKRIIWDSRKGFIISNATYKEIGLLTCEATVNGHLYKTNYLTHRQTNTIIDVVLSPSHGIELSVGEKLVLNCTARTELNVGIDFNWEYPSSKHQHKKLVNRDLKTQSGSEMKKFLSTLTIDGVTRSDQGLYTCAASSGLMTKKNSTFVRVHEK

SEQ ID NO: 53 - protein, 455 aa, synthetic construct
  REGION 1..455: note = source = /note="Description of Artificial Sequence: Synthetic polypeptide"
SDTGRPFVEMYSEIPEIIHMTEGRELVIPCRVTSPNITVTLKKFPLDTLIPDGKRIIWDSRKGFIISNATYKEIGLLTCEATVNGHLYKTNYLTHRQTNTIIDVVLSPSHGIELSVGEKLVLNCTARTELNVGIDFNWEYPSSKHQHKKLVNRDLKTQSGSEMKKFLSTLTIDGVTRSDQGLYTCAASSGLMTKKNSTFVRVHEKGGGGSGGGGSGGGGSGGGGSGGGGSGGGGSGGGGSGGGGSGGGGSSDTGRPFVEMYSEIPEIIHMTEGRELVIPCRVTSPNITVTLKKFPLDTLIPDGKRIIWDSRKGFIISNATYKEIGLLTCEATVNGHLYKTNYLTHRQTNTIIDVVLSPSHGIELSVGEKLVLNCTARTELNVGIDFNWEYPSSKHQHKKLVNRDLKTQSGSEMKKFLSTLTIDGVTRSDQGLYTCAASSGLMTKKNSTFVRVHEK

SEQ ID NO: 54 - protein, 470 aa, synthetic construct
  REGION 1..470: note = source = /note="Description of Artificial Sequence: Synthetic polypeptide"
SDTGRPFVEMYSEIPEIIHMTEGRELVIPCRVTSPNITVTLKKFPLDTLIPDGKRIIWDSRKGFIISNATYKEIGLLTCEATVNGHLYKTNYLTHRQTNTIIDVVLSPSHGIELSVGEKLVLNCTARTELNVGIDFNWEYPSSKHQHKKLVNRDLKTQSGSEMKKFLSTLTIDGVTRSDQGLYTCAASSGLMTKKNSTFVRVHEKGGGGSGGGGSGGGGSGGGGSGGGGSGGGGSGGGGSGGGGSGGGGSGGGGSGGGGSGGGGSSDTGRPFVEMYSEIPEIIHMTEGRELVIPCRVTSPNITVTLKKFPLDTLIPDGKRIIWDSRKGFIISNATYKEIGLLTCEATVNGHLYKTNYLTHRQTNTIIDVVLSPSHGIELSVGEKLVLNCTARTELNVGIDFNWEYPSSKHQHKKLVNRDLKTQSGSEMKKFLSTLTIDGVTRSDQGLYTCAASSGLMTKKNSTFVRVHEK

SEQ ID NO: 55 - protein, 434 aa, synthetic construct
  REGION 1..434: note = source = /note="Description of Artificial Sequence: Synthetic polypeptide"
SDTGRPFVEMYSEIPEIIHMTEGRELVIPCRVTSPNITVTLKKFPLDTLIPDGKRIIWDSRKGFIISNATYKEIGLLTCEATVNGHLYKTNYLTHRQTNTIIDVVLSPSHGIELSVGEKLVLNCTARTELNVGIDFNWEYPSSKHQHKKLVNRDLKTQSGSEMKKFLSTLTIDGVTRSDQGLYTCAASSGLMTKKNSTFVRVHEKDKTHTCPPCPAPELLGGPSVFLFPPKPKDTLMISRTPEVTCVVVDVSHEDPEVKFMWYVDGSSVEVHNAKTKPREEQYNSTYRVVSVLTVLHQDWLNGKEYKCKVSNKALPAPIEKTISKAKGQPREPQVYTLPPSRDELTKNQVSLTCLVKGFYPSDIAVEWESNGQPENNYKTTPPVLDSDGSFFLYSKLTVDKSRWQQGNVFSCSVMHEALHNHYTQKSLSLSPGK

SEQ ID NO: 56 - protein, 6 aa, synthetic construct
  REGION 1..6: note = source = /note="Description of Artificial Sequence: Synthetic peptide"
IIWDSR

SEQ ID NO: 57 - protein, 17 aa, synthetic construct
  REGION 1..17: note = source = /note="Description of Artificial Sequence: Synthetic peptide"
EIGLLTCEATVNGHLYK

SEQ ID NO: 58 - protein, 23 aa, synthetic construct
  REGION 1..23: note = source = /note="Description of Artificial Sequence: Synthetic peptide"
QTNTIIDVVLSPSHGIELSVGEK

SEQ ID NO: 59 - protein, 21 aa, synthetic construct
  REGION 1..21: note = source = /note="Description of Artificial Sequence: Synthetic peptide"
TELNVGIDFNWEYPSSKHQHK

SEQ ID NO: 60 - protein, 16 aa, synthetic construct
  REGION 1..16: note = source = /note="Description of Artificial Sequence: Synthetic peptide"
DKTHTCPPCPAPELLG

SEQ ID NO: 61 - protein, 7 aa, synthetic construct
  REGION 1..7: note = source = /note="Description of Artificial Sequence: Synthetic peptide"
TNYLTHR

SEQ ID NO: 62 - protein, 17 aa, synthetic construct
  REGION 1..17: note = source = /note="Description of Artificial Sequence: Synthetic peptide"
EIGLLTCEATVNGHLYK

SEQ ID NO: 63 - protein, 23 aa, synthetic construct
  REGION 1..23: note = source = /note="Description of Artificial Sequence: Synthetic peptide"
QTNTIIDVVLSPSHGIELSVGEK

SEQ ID NO: 64 - protein, 24 aa, synthetic construct
  REGION 1..24: note = source = /note="Description of Artificial Sequence: Synthetic peptide"
SDTGRPFVEMYSEIPEIIHMTEGR

SEQ ID NO: 65 - protein, 24 aa, synthetic construct
  REGION 1..24: note = source = /note="Description of Artificial Sequence: Synthetic peptide"
SDTGRPFVEMYSEIPEIIHMTEGR

SEQ ID NO: 66 - protein, 8 aa, synthetic construct
  REGION 1..8: note = source = /note="Description of Artificial Sequence: Synthetic peptide"
TQSGSEMK

SEQ ID NO: 67 - protein, 17 aa, synthetic construct
  REGION 1..17: note = source = /note="Description of Artificial Sequence: Synthetic peptide"
SDQGLYTCAASSGLMTK

SEQ ID NO: 68 - protein, 24 aa, synthetic construct
  REGION 1..24: note = source = /note="Description of Artificial Sequence: Synthetic peptide"
SDTGRPFVEMYSEIPEIIHMTEGR

SEQ ID NO: 69 - protein, 10 aa, synthetic construct
  REGION 1..10: note = source = /note="Description of Artificial Sequence: Synthetic peptide"
GFIISNATYK

SEQ ID NO: 70 - protein, 12 aa, synthetic construct
  REGION 1..12: note = source = /note="Description of Artificial Sequence: Synthetic peptide"
KFPLDTLIPDGK

SEQ ID NO: 71 - protein, 12 aa, synthetic construct
  REGION 1..12: note = source = /note="Description of Artificial Sequence: Synthetic peptide"
FLSTLTIDGVTR

SEQ ID NO: 72 - protein, 165 aa, synthetic construct
  REGION 1..165: note = source = /note="Description of Artificial Sequence: Synthetic polypeptide"
APMAEGGGQNHHEVVKFMDVYQRSYCHPIETLVDIFQEYPDEIEYIFKPSCVPLMRCGGCCNDEGLECVPTEESNITMQIMRIKPHQGQHIGEMSFLQHNKCECRPKKDRARQENPCGPCSERRKHLFVQDPQTCKCSCKNTDSRCKARQLELNERTCRCDKPRR

SEQ ID NO: 73 - protein, 451 aa, synthetic construct
  REGION 1..451: note = source = /note="Description of Artificial Sequence: Synthetic polypeptide"
EVQLVESGGDLVKPGGSLKLSCAASGFTFSSSGMSWVRQTPDKRLEWVATITSGGSYTYYPDSVKGRFTISRDNAKNTLYLQMSSLKSEDTAMFYCARLGNYGGYYAMDYWGQGTSVTVSSASTKGPSVFPLAPSSKSTSGGTAALGCLVKDYFPEPVTVSWNSGALTSGVHTFPAVLQSSGLYSLSSVVTVPSSSLGTQTYICNVNHKPSNTKVDKKVEPKSCDKTHTCPPCPAPELLGGPSVFLFPPKPKDTLMISRTPEVTCVVVDVSHEDPEVKFNWYVDGVEVHNAKTKPREEQYNSTYRVVSVLTVLHQDWLNGKEYKCKVSNKALPAPIEKTISKAKGQPREPQVYTLPPSRDELTKNQVSLTCLVKGFYPSDIAVEWESNGQPENNYKTTPPVLDSDGSFFLYSKLTVDKSRWQQGNVFSCSVMHEALHNHYTQKSLSLSPGK

SEQ ID NO: 74 - protein, 213 aa, synthetic construct
  REGION 1..213: note = source = /note="Description of Artificial Sequence: Synthetic polypeptide"
DIQMTQSPSSLSASLGGKVTITCTTSQDSNNYIAWYQHKPGKGPRLLIHYASTLQPGIPSRFSGSGSGRDYSFSISNLEPEDIATYFCLQYDYLWTFGGGTKLELKRTVAAPSVFIFPPSDEQLKSGTASVVCLLNNFYPREAKVQWKVDNALQSGNSQESVTEQDSKDSTYSLSSTLTLSKADYEKHKVYACEVTHQGLSSPVTKSFNRGEC

SEQ ID NO: 75 - protein, 451 aa, synthetic construct
  REGION 1..451: note = source = /note="Description of Artificial Sequence: Synthetic polypeptide"
EVQLVESGGDLVKPGGSLKLSCAASGFTFSDSGMSWVRQTPDKRLEWVATISSGGGYTYYSDSVEGRFTISRDNANNTLFLQMSSLKSEDTAMFYCARLGNYGGYYGMDYWGQGTSVTVSSASTKGPSVFPLAPSSKSTSGGTAALGCLVKDYFPEPVTVSWNSGALTSGVHTFPAVLQSSGLYSLSSVVTVPSSSLGTQTYICNVNHKPSNTKVDKKVEPKSCDKTHTCPPCPAPELLGGPSVFLFPPKPKDTLMISRTPEVTCVVVDVSHEDPEVKFNWYVDGVEVHNAKTKPREEQYNSTYRVVSVLTVLHQDWLNGKEYKCKVSNKALPAPIEKTISKAKGQPREPQVYTLPPSRDELTKNQVSLTCLVKGFYPSDIAVEWESNGQPENNYKTTPPVLDSDGSFFLYSKLTVDKSRWQQGNVFSCSVMHEALHNHYTQKSLSLSPGK

SEQ ID NO: 76 - protein, 213 aa, synthetic construct
  REGION 1..213: note = source = /note="Description of Artificial Sequence: Synthetic polypeptide"
DIQMTQSPSSLSASLGGKVTITCKTSQDSNKYIAWYQHKPGKGPRLLIHYTSTLQPGIPSRFSGSGSGRDYSFSISNLEPEDIATYYCLQYDNLWTFGGGTKLEIKRTVAAPSVFIFPPSDEQLKSGTASVVCLLNNFYPREAKVQWKVDNALQSGNSQESVTEQDSKDSTYSLSSTLTLSKADYEKHKVYACEVTHQGLSSPVTKSFNRGEC

SEQ ID NO: 77 - protein, 445 aa, synthetic construct
  REGION 1..445: note = source = /note="Description of Artificial Sequence: Synthetic polypeptide"
EVQLVESGGDLVKPGGSLKLSCAASGFTFSSSGMSWVRQTPDKRLEWVATITSGGSYTYYPDSVKGRFTISRDNAKNTLYLQMSSLKSEDTAMFYCARLGNYGGYYAMDYWGQGTSVTVSSAKTTPPSVYPLAPGSAAQTNSMVTLGCLVKGYFPEPVTVTWNSGSLSSGVHTFPAVLQSDLYTLSSSVTVPSSTWPSETVTCNVAHPASSTKVDKKIVPRDCGCKPCICTVPEVSSVFIFPPKPKDVLTITLTPKVTCVVVDISKDDPEVQFSWFVDDVEVHTAQTQPREEQFNSTFRSVSELPIMHQDWLNGKEFKCRVNSAAFPAPIEKTISKTKGRPKAPQVYTIPPPKEQMAKDKVSLTCMITDFFPEDITVEWQWNGQPAENYKNTQPIMDTDGSYFVYSKLNVQKSNWEAGNTFTCSVLHEGLHNHHTEKSLSHSPGK

SEQ ID NO: 78 - protein, 213 aa, synthetic construct
  REGION 1..213: note = source = /note="Description of Artificial Sequence: Synthetic polypeptide"
DIQMTQSPSSLSASLGGKVTITCTTSQDSNNYIAWYQHKPGKGPRLLIHYASTLQPGIPSRFSGSGSGRDYSFSISNLEPEDIATYFCLQYDYLWTFGGGTKLELKRADAAPTVSIFPPSSEQLTSGGASVVCFLNNFYPKDINVKWKIDGSERQNGVLNSWTDQDSKDSTYSMSSTLTLTKDEYERHNSYTCEATHKTSTSPIVKSFNRGEC

SEQ ID NO: 79 - protein, 445 aa, synthetic construct
  REGION 1..445: note = source = /note="Description of Artificial Sequence: Synthetic polypeptide"
EVQLVESGGDLVKPGGSLKLSCAASGFTFSDSGMSWVRQTPDKRLEWVATISSGGGYTYYSDSVEGRFTISRDNANNTLFLQMSSLKSEDTAMFYCARLGNYGGYYGMDYWGQGTSVTVSSAKTTPPSVYPLAPGSAAQTNSMVTLGCLVKGYFPEPVTVTWNSGSLSSGVHTFPAVLQSDLYTLSSSVTVPSSTWPSETVTCNVAHPASSTKVDKKIVPRDCGCKPCICTVPEVSSVFIFPPKPKDVLTITLTPKVTCVVVDISKDDPEVQFSWFVDDVEVHTAQTQPREEQFNSTFRSVSELPIMHQDWLNGKEFKCRVNSAAFPAPIEKTISKTKGRPKAPQVYTIPPPKEQMAKDKVSLTCMITDFFPEDITVEWQWNGQPAENYKNTQPIMDTDGSYFVYSKLNVQKSNWEAGNTFTCSVLHEGLHNHHTEKSLSHSPGK

SEQ ID NO: 80 - protein, 200 aa, synthetic construct
  REGION 1..200: note = source = /note="Description of Artificial Sequence: Synthetic polypeptide"
DIQMTQSPSSLSASLGGKVTITCKTSQDSNKYIAWYQHKPGKGPRLLIHYTSTLQPGIPSRFSGSGSGRDYSFSISNLEPEDIATYYCLQYDNLWTFGGGTKLEIKRADAAPTVSIFPPSSEQLTSGGASVVCFLNNFYPKDINVKWKIDGSERQNGVLNSWTDQDSKDSTYSMSSTLTLTKDEYERHNSYTCEATHKTS

SEQ ID NO: 81 - protein, 7 aa, synthetic construct
  REGION 1..7: note = source = /note="Description of Artificial Sequence: Synthetic peptide"
ELVIPCR

SEQ ID NO: 82 - protein, 8 aa, synthetic construct
  REGION 1..8: note = source = /note="Description of Artificial Sequence: Synthetic peptide"
LVLNCTAR

SEQ ID NO: 83 - protein, 14 aa, synthetic construct
  REGION 1..14: note = source = /note="Description of Artificial Sequence: Synthetic peptide"
THTCPPCPAPELLG

SEQ ID NO: 84 - protein, 24 aa, synthetic construct
  REGION 1..24: note = source = /note="Description of Artificial Sequence: Synthetic peptide"
ELVIPCREIGLLTCEATVNGHLYK

SEQ ID NO: 85 - protein, 26 aa, synthetic construct
  VARIANT 26: note = /replace=" "
  SITE 1..26: note = /note="Variant residues given in the sequence have no preference with respect to those in the annotations for variant positions"
  REGION 1..26: note = source = /note="Description of Artificial Sequence: Synthetic peptide"
LVLNCTARSDQGLYTCAASSGLMTKK

SEQ ID NO: 86 - protein, 28 aa, synthetic construct
  VARIANT 28: note = /replace=" "
  SITE 1..28: note = /note="Variant residues given in the sequence have no preference with respect to those in the annotations for variant positions"
  REGION 1..28: note = source = /note="Description of Artificial Sequence: Synthetic peptide"
THTCPPCPAPELLGTHTCPPCPAPELLG

SEQ ID NO: 87 - protein, 17 aa, synthetic construct
  REGION 1..17: note = source = /note="Description of Artificial Sequence: Synthetic peptide"
EIGLLTCEATVNGHLYK

SEQ ID NO: 88 - protein, 23 aa, synthetic construct
  REGION 1..23: note = source = /note="Description of Artificial Sequence: Synthetic peptide"
QTNTIIDVVLSPSHGIELSVGEK

SEQ ID NO: 89 - protein, 24 aa, synthetic construct
  REGION 1..24: note = source = /note="Description of Artificial Sequence: Synthetic peptide"
SDTGRPFVEMYSEIPEIIHMTEGR

SEQ ID NO: 90 - protein, 24 aa, synthetic construct
  REGION 1..24: note = source = /note="Description of Artificial Sequence: Synthetic peptide"
SDTGRPFVEMYSEIPEIIHMTEGR

SEQ ID NO: 91 - protein, 54 aa, synthetic construct
  REGION 1..54: note = source = /note="Description of Artificial Sequence: Synthetic polypeptide"
GGGGSGGGGSGGGGSGGGGSGGGGSGGGGSSDTGRPFVEMYSEIPEIIHMTEGR

SEQ ID NO: 92 - protein, 54 aa, synthetic construct; identical to SEQ ID NO: 91
  REGION 1..54: note = source = /note="Description of Artificial Sequence: Synthetic polypeptide"

SEQ ID NO: 93 - protein, 8 aa, synthetic construct
  REGION 1..8: note = source = /note="Description of Artificial Sequence: Synthetic peptide"
TQSGSEMK

SEQ ID NO: 94 - protein, 17 aa, synthetic construct
  REGION 1..17: note = source = /note="Description of Artificial Sequence: Synthetic peptide"
SDQGLYTCAASSGLMTK

SEQ ID NO: 95 - protein, 14 aa, synthetic construct
  REGION 1..14: note = source = /note="Description of Artificial Sequence: Synthetic peptide"
THTCPPCPAPELLG

SEQ ID NO: 96 - protein, 23 aa, synthetic construct
  REGION 1..23: note = source = /note="Description of Artificial Sequence: Synthetic peptide"
QTNTIIDVVLSPSHGIELSVGEK

SEQ ID NO: 97 - protein, 7 aa, synthetic construct
  REGION 1..7: note = source = /note="Description of Artificial Sequence: Synthetic peptide"
  REGION 1..7: note = source = /note="See specification as filed for detailed description of substitutions and preferred embodiments"
TNYLTHR

SEQ ID NO: 98 - protein, 54 aa, synthetic construct; identical to SEQ ID NO: 91
  REGION 1..54: note = source = /note="Description of Artificial Sequence: Synthetic polypeptide"

SEQ ID NO: 99 - protein, 24 aa, synthetic construct
  REGION 1..24: note = source = /note="Description of Artificial Sequence: Synthetic peptide"
SDTGRPFVEMYSEIPEIIHMTEGR

SEQ ID NO: 100 - protein, 12 aa, synthetic construct
  VARIANT 1: note = /replace=" "
  SITE 1..12: note = /note="Variant residues given in the sequence have no preference with respect to those in the annotations for variant positions"
  REGION 1..12: note = source = /note="Description of Artificial Sequence: Synthetic peptide"
RVTSPNITVTLK

SEQ ID NO: 101 - protein, 11 aa, synthetic construct
  VARIANT 1: note = /replace=" "
  SITE 1..11: note = /note="Variant residues given in the sequence have no preference with respect to those in the annotations for variant positions"
  REGION 1..11: note = source = /note="Description of Artificial Sequence: Synthetic peptide"
KGFIISNATYK

SEQ ID NO: 102 - protein, 9 aa, synthetic construct
  VARIANT 1: note = /replace=" "
  SITE 1..9: note = /note="Variant residues given in the sequence have no preference with respect to those in the annotations for variant positions"
  REGION 1..9: note = source = /note="Description of Artificial Sequence: Synthetic peptide"
KLVLNCTAR

SEQ ID NO: 103 - protein, 7 aa, synthetic construct
  VARIANT 1: note = /replace=" "
  SITE 1..7: note = /note="Variant residues given in the sequence have no preference with respect to those in the annotations for variant positions"
  REGION 1..7: note = source = /note="Description of Artificial Sequence: Synthetic peptide"
KNSTFVR